European Patent Specification EP 3 583 127 B1, published November 20, 2024. Title: ANTI-PROGRAMMED DEATH-LIGAND 1 (PD-L1) ANTIBODIES AND THERAPEUTIC USES THEREOF. Applicant: Shenzhen RunShin Bioscience ZHANG, YING. The sequence listing filed with the application follows.

SEQUENCE LISTING (20 sequences)

SEQ ID NO: 1 - DNA, 360 bp, Mouse
tctgatgtgcagcttcaggagtcgggacctggcctggtgaaaccttctcagtctctgtccctcacctgctctgtcactggctactctatcaccagtgattatgcctggaactggatccggcagtttccaggagacacactggagtggatgggctacataaactacagtggtagctctacctacaacccatctctcataagtcgactctctatcactcgagacacatccaagaaccagttcttcctgcagttgaattctgtgacttctgaggacacagccacatattactgtgcaagaggccctgactgggactggtactttgactactggggccaaggcaccactctcacagtctcctca

SEQ ID NO: 2 - protein, 120 aa, Mouse
SDVQLQESGPGLVKPSQSLSLTCSVTGYSITSDYAWNWIRQFPGDTLEWMGYINYSGSSTYNPSLISRLSITRDTSKNQFFLQLNSVTSEDTATYYCARGPDWDWYFDYWGQGTTLTVSS

SEQ ID NO: 3 - DNA, 318 bp, Mouse
gatattgtgctaactcagtctccagccaccctgtctgtgactccaggagatagcgtcagtctttcctgcagggccagccaaagtattagcaacaacctacactggtatcaacaaaaatcacatgagtctccaaggcttctcatcaagtacgcttcccagtccatctctgggatcccctccaggttcagtggcagtggatcagggaccgatttcactctcagtatcaacggtgtggagactgaagattttggaatgtatttctgtcaacagactaacagctggccgacgttcggtggaggcaccaaactggaaatcaaa

SEQ ID NO: 4 - protein, 106 aa, Mouse
DIVLTQSPATLSVTPGDSVSLSCRASQSISNNLHWYQQKSHESPRLLIKYASQSISGIPSRFSGSGSGTDFTLSINGVETEDFGMYFCQQTNSWPTFGGGTKLEIK

SEQ ID NO: 5 - DNA, 360 bp, Mouse
gaggatgtgcagcttcaggagtcgggacctggcctggtgaaaccttctcagtctctgtccctcacctgctctgtcactggctactctatctctagtgattatgcctggaactggatccggcagtttggcggagacacactggagtggatgggctacataaactacagtggtagctctacctacaacgggtctctcataagtcgactctcttctactcgagacacatccaagaaccagttcttcctgcagttgaattctgtgacttctgaggacacagccacatattactgtgcaagaggcccttcaggggactggtacaacgactactggggccaaggcaccactctcacagtctcctca

SEQ ID NO: 6 - protein, 120 aa, Mouse
EDVQLQESGPGLVKPSQSLSLTCSVTGYSISSDYAWNWIRQFGGDTLEWMGYINYSGSSTYNGSLISRLSSTRDTSKNQFFLQLNSVTSEDTATYYCARGPSGDWYNDYWGQGTTLTVSS

SEQ ID NO: 7 - DNA, 318 bp, Mouse
gatattgtgctaactcagtctccagccgacctgtctgtgactccaggagatagcgtcagtctttcctgcagggccagccaaagtattagctcaaacctacactggtatcaacaaaaatcacatgagtctccaaggcttctcatcaagtacgcttcccagtccggctctgggatcccctccaggttcagtggcagtggatcagggaccgatttcactctcagtatcaacggtgtggagactgaagattttggaatgtatttctgtcaacagactaacatttggggcacgttcggtggaggcaccaaactggaaatcaaa

SEQ ID NO: 8 - protein, 106 aa, Mouse
DIVLTQSPADLSVTPGDSVSLSCRASQSISSNLHWYQQKSHESPRLLIKYASQSGSGIPSRFSGSGSGTDFTLSINGVETEDFGMYFCQQTNIWGTFGGGTKLEIK

SEQ ID NO: 9 - protein, 9 aa, Mouse
GYSITSDYA

SEQ ID NO: 10 - protein, 10 aa, Mouse
SGSSTYNPSL

SEQ ID NO: 11 - protein, 10 aa, Mouse
GPDWDWYFDY

SEQ ID NO: 12 - protein, 6 aa, Mouse
QSISNN

SEQ ID NO: 13 - protein, 6 aa, Mouse
ASQSIS

SEQ ID NO: 14 - protein, 8 aa, Mouse
QQTNSWPT

SEQ ID NO: 15 - protein, 9 aa, Mouse
GYSISSDYA

SEQ ID NO: 16 - protein, 10 aa, Mouse
SGSSTYNGSL

SEQ ID NO: 17 - protein, 10 aa, Mouse
GPSGDWYNDY

SEQ ID NO: 18 - protein, 6 aa, Mouse
QSISSN

SEQ ID NO: 19 - protein, 6 aa, Mouse
ASQSGS

SEQ ID NO: 20 - protein, 8 aa, Mouse
QQTNIWGT